European Patent Application EP 4 299 742 A1, published January 3, 2024. Title: COMBINATION THERAY FOR MELANOMA. Applicant: Université de Strasbourg Institut National de la Santé et de la Recherche Médicale Centre National de la Recherche Scientifique Katholieke Universiteit Leuven. The sequence listing filed with the application follows.

SEQUENCE LISTING (13 sequences)

SEQ ID NO: 1 - DNA, 15 bp, Artificial Sequence
  Antisense ASO-CTR
aacacgtctatacgc

SEQ ID NO: 2 - DNA, 16 bp, Artificial Sequence
  Antisense ASO1-LINC00518
ccgacctgaattgcaa

SEQ ID NO: 3 - DNA, 16 bp, Artificial Sequence
  Antisense ASO2-LINC00518
gtagaggctagaactg

SEQ ID NO: 4 - DNA, 14 bp, Artificial Sequence
  Antisense ASO-SAMMSON
gtgtgaacttggct

SEQ ID NO: 5 - DNA, 16 bp, Artificial Sequence
  Gapmer Gap1-LINC00518
  misc_feature (1)..(3): LNA (2',4'-methylene bridged sugar moiety)
  misc_feature (1)..(15): phosphothiorate internucleotide linkage between each nucleotide, in lieu of phosphodiester linkage
  modified_base (5)..(6): m5c
  misc_feature (14)..(16): LNA (2',4'-methylene bridged sugar moiety)
ccgacctgaattgcaa

SEQ ID NO: 6 - DNA, 16 bp, Artificial Sequence
  Gapmer Gap2-LINC00518
  misc_feature (1)..(3): LNA (2',4'-methylene bridged sugar moiety)
  misc_feature (1)..(15): phosphothiorate internucleotide linkage between each nucleotide, in lieu of phosphodiester linkage
  modified_base (8)..(8): m5c
  misc_feature (14)..(16): LNA (2',4'-methylene bridged sugar moiety)
gtagaggctagaactg

SEQ ID NO: 7 - DNA, 14 bp, Artificial Sequence
  Gapmer Gap-SAMMSON
  misc_feature (1)..(3): LNA (2',4'-methylene bridged sugar moiety)
  misc_feature (1)..(13): phosphothiorate internucleotide linkage between each nucleotide, in lieu of phosphodiester linkage
  modified_base (8)..(8): m5c
  misc_feature (12)..(14): LNA (2',4'-methylene bridged sugar moiety)
gtgtgaacttggct

SEQ ID NO: 8 - DNA, 21 bp, Artificial Sequence
  RNAi i-CTR
attacgtctgtcatgaacctc

SEQ ID NO: 9 - DNA, 21 bp, Artificial Sequence
  RNAi i-LINC00518
ttcactaaggttccatctagc

SEQ ID NO: 10 - RNA, 21 nt, Artificial Sequence
  RNAi i-SAMMSON
gucgcuagacauuugaggaaa

SEQ ID NO: 11 - DNA, 20 bp, Artificial Sequence
  sgRNA sg1-LINC00518
ccgagagagaggactctctg

SEQ ID NO: 12 - DNA, 20 bp, Artificial Sequence
  sgRNA sg2-LINC00518
tgttactaatgagaccgctg

SEQ ID NO: 13 - DNA, 20 bp, Artificial Sequence
  sgRNA sg3-LINC00518
actgatacacactataaacg